European Patent Specification EP 4 065 117 B1, published June 19, 2024. Title: LACTATE ENHANCING COMPOUNDS AND USES THEREOF IN GLUT1 DEFICIENCY SYNDROME. Applicant: GLIAPHARM SA. The sequence listing filed with the application follows.

SEQUENCE LISTING (2 sequences)

SEQ ID NO: 1 - RNA, 19 nt, Artificial sequence
  Scramble siRNA
agguaguguaaucgccuug

SEQ ID NO: 2 - RNA, 19 nt, Artificial sequence
  GLUT1 siRNA
guauagauggaagauauuu